European Patent Application EP 4 375 372 A1, published May 29, 2024. Title: ANTIBACTERIAL PEPTIDE P104 AND LYSIN LYSP53 WITH BROAD-SPECTRUM LYTIC ACTIVITY, AND APPLICATIONS THEREOF. Applicant: Wuhan Institute of Virology, Chinese Academy of Sciences. The sequence listing filed with the application follows.

SEQUENCE LISTING (6 sequences)

SEQ ID NO: 1 - protein, 33 aa, antibacterial peptide (P104)
MTMTTKRIFEHMRPNLTDSQVQALYKLMEKGAD

SEQ ID NO: 2 - protein, 209 aa, lysin (LysP53)
MTMTTKRIFEHMRPNLTDSQVQALYKLMEKGADLDTIAQFAGVSPLVSTADVKQPSGFKFSQTSLKRLEGVNPKLVQVVNRALEISKEDFMVIEGVRTKESAWANWGKGRTAAQCQAAGVPTKYAQPSLAKVTWLTDPLKSKHMTGHAVDLAPIPLDWNDLKRFDLMAQAMFQASAELNIPIRWGADWDNDGVFREKGETDSPHFELAG

SEQ ID NO: 3 - DNA, 99 bp, gene of antibacterial peptide (P104)
atgacgatgacaacaaaacgtattttcgagcatatgcgtccgaatctcacggactcacaagtacaagcgctgtacaagctcatggaaaaaggtgcagac

SEQ ID NO: 4 - DNA, 630 bp, gene of lysin (LysP53)
atgacgatgacaacaaaacgtattttcgagcatatgcgtccgaatctcacggactcacaagtacaagcgctgtacaagctcatggaaaaaggtgcagaccttgacaccattgcacagttcgcaggggtatcgccgttagtatccacagccgacgtaaaacagccgagcggctttaagttcagccaaacatcattaaaacgacttgagggcgtaaatcctaagttagtgcaagtggttaatcgtgccttggaaatcagtaaagaggatttcatggtgatcgaaggagtccgcactaaggaaagtgcatgggccaactggggtaaaggacgcacggcggcacagtgccaagctgcaggagtgccgaccaagtatgcccaaccaagtctggctaaggtgacatggctcacagatccacttaaaagcaaacacatgacaggccacgccgtggacctagctccaatcccactggactggaacgaccttaaacgattcgacctaatggcccaagcgatgtttcaagcatccgccgagttaaatatcccgattcgttggggtgccgactgggacaacgatggcgtattccgtgaaaaaggtgagactgacagcccacactttgaattggcggggtga

SEQ ID NO: 5 - DNA, 46 bp, Artificial Sequence
ctttaagaaggagatataccatggatgacgatgacaacaaaacgta

SEQ ID NO: 6 - DNA, 47 bp, Artificial Sequence
tggtggtggtggtggtgctcgagccccgccaattcaaagtgtgggct